European Patent Application EP 4 682 173 A1, published January 21, 2026. Title: Production method of radioisotope-labeled antibody, radioisotope-labeled antibody and radiopharmaceutical. Applicant: Kagoshima University. Application WO. The sequence listing filed with the application follows.

SEQUENCE LISTING (168 sequences)

SEQ ID NO: 1 - protein, 13 aa, synthetic construct
  REGION 1..13: note = Fc binding peptide
  SITE 6: note = MISC_FEATURE - X is K, C, D, E, R, V, F, L, 2-Aminooctanedioic acid, Dpr, Orn,AcOrn, AcDab, Dab, Nle, Nva, Tle, Ala(t-Bu), or Cha
DCAYHXGELVWCT

SEQ ID NO: 2 - protein, 17 aa, synthetic construct
  REGION 1..17: note = IgG binding peptide
  SITE 8: note = MISC_FEATURE - X is K, C, D, E, R, V, F, L, 2-Aminooctanedioic acid, Dpr, Orn,AcOrn, AcDab, Dab, Nle, Nva, Tle, Ala(t-Bu), or Cha
GPDCAYHXGELVWCTFH

SEQ ID NO: 3 - protein, 13 aa, synthetic construct
  REGION 1..13: note = IgG binding peptide
  SITE 6: note = MISC_FEATURE - X is K, C, D, E, R, V, F, L, 2-Aminooctanedioic acid, Dpr, Orn,AcOrn, AcDab, Dab, Nle, Nva, Tle, Ala(t-Bu), or Cha
RCAYHXGELVWCS

SEQ ID NO: 4 - protein, 17 aa, synthetic construct
  REGION 1..17: note = IgG binding peptide
  SITE 8: note = MISC_FEATURE - X is K, C, D, E, R, V, F, L, 2-Aminooctanedioic acid, Dpr, Orn,AcOrn, AcDab, Dab, Nle, Nva, Tle, Ala(t-Bu), or Cha
GPRCAYHXGELVWCSFH

SEQ ID NO: 5 - protein, 17 aa, synthetic construct
  REGION 1..17: note = IgG binding peptide
  SITE 8: note = MISC_FEATURE - X is K, C, D, E, R, V, F, L, 2-Aminooctanedioic acid, Dpr, Orn,AcOrn, AcDab, Dab, Nle, Nva, Tle, Ala(t-Bu), or Cha
SPDCAYHXGELVWCTFH

SEQ ID NO: 6 - protein, 17 aa, synthetic construct
  REGION 1..17: note = IgG binding peptide
  SITE 8: note = MISC_FEATURE - X is K, C, D, E, R, V, F, L, 2-Aminooctanedioic acid, Dpr, Orn,AcOrn, AcDab, Dab, Nle, Nva, Tle, Ala(t-Bu), or Cha
GDDCAYHXGELVWCTFH

SEQ ID NO: 7 - protein, 17 aa, synthetic construct
  REGION 1..17: note = IgG binding peptide
  SITE 8: note = MISC_FEATURE - X is K, C, D, E, R, V, F, L, 2-Aminooctanedioic acid, Dpr, Orn,AcOrn, AcDab, Dab, Nle, Nva, Tle, Ala(t-Bu), or Cha
GPSCAYHXGELVWCTFH

SEQ ID NO: 8 - protein, 17 aa, synthetic construct
  REGION 1..17: note = IgG binding peptide
  SITE 8: note = MISC_FEATURE - X is K, C, D, E, R, V, F, L, 2-Aminooctanedioic acid, Dpr, Orn,AcOrn, AcDab, Dab, Nle, Nva, Tle, Ala(t-Bu), or Cha
GPDCAYHXGELVWCSFH

SEQ ID NO: 9 - protein, 17 aa, synthetic construct
  REGION 1..17: note = IgG binding peptide
  SITE 8: note = MISC_FEATURE - X is K, C, D, E, R, V, F, L, 2-Aminooctanedioic acid, Dpr, Orn,AcOrn, AcDab, Dab, Nle, Nva, Tle, Ala(t-Bu), or Cha
GPDCAYHXGELVWCTHH

SEQ ID NO: 10 - protein, 17 aa, synthetic construct
  REGION 1..17: note = IgG binding peptide
  SITE 8: note = MISC_FEATURE - X is K, C, D, E, R, V, F, L, 2-Aminooctanedioic acid, Dpr, Orn,AcOrn, AcDab, Dab, Nle, Nva, Tle, Ala(t-Bu), or Cha
GPDCAYHXGELVWCTFY

SEQ ID NO: 11 - protein, 17 aa, synthetic construct
  REGION 1..17: note = IgG binding peptide
  SITE 8: note = MISC_FEATURE - X is K,C, D, E, R, V, F, L, 2-Aminooctanedioic acid, Dpr, Orn,AcOrn, AcDab, Dab, Nle, Nva, Tle, Ala(t-Bu), or Cha
SPDCAYHXGELVWCTFY

SEQ ID NO: 12 - protein, 17 aa, synthetic construct
  REGION 1..17: note = IgG binding peptide
  SITE 8: note = MISC_FEATURE - X is K, C, D, E, R, V, F, L, 2-Aminooctanedioic acid, Dpr, Orn,AcOrn, AcDab, Dab, Nle, Nva, Tle, Ala(t-Bu), or Cha
SDDCAYHXGELVWCTFY

SEQ ID NO: 13 - protein, 17 aa, synthetic construct
  REGION 1..17: note = IgG binding peptide
  SITE 8: note = MISC_FEATURE - X is K, C, D, E, R, V, F, L, 2-Aminooctanedioic acid, Dpr, Orn,AcOrn, AcDab, Dab, Nle, Nva, Tle, Ala(t-Bu), or Cha
RGNCAYHXGQLVWCTYH

SEQ ID NO: 14 - protein, 17 aa, synthetic construct
  REGION 1..17: note = IgG binding peptide
  SITE 2: note = MISC_FEATURE - X is homocysteine
  SITE 8: note = MISC_FEATURE - X is K, C, D, E, R, V, F, L, 2-Aminooctanedioic acid, Dpr, Orn,AcOrn, AcDab, Dab, Nle, Nva, Tle, Ala(t-Bu), or Cha
  SITE 16: note = MISC_FEATURE - X is homocysteine
GXDCAYHXGELVWCTXH

SEQ ID NO: 15 - protein, 19 aa, synthetic construct
  REGION 1..19: note = IgG binding peptide
  SITE 10: note = MISC_FEATURE - X is K, C, D, E, R, V, F, L, 2-Aminooctanedioic acid, Dpr, Orn,AcOrn, AcDab, Dab, Nle, Nva, Tle, Ala(t-Bu), or Cha
RRGPDCAYHXGELVWCTFH

SEQ ID NO: 16 - protein, 13 aa, synthetic construct
  REGION 1..13: note = IgG binding peptide
  SITE 6: note = MISC_FEATURE - X is K, C, D, E, R, V, F, L, 2-Aminooctanedioic acid, Dpr, Orn,AcOrn, AcDab, Dab, Nle, Nva, Tle, Ala(t-Bu), or Cha
DCTYHXGNLVWCT

SEQ ID NO: 17 - protein, 13 aa, synthetic construct
  REGION 1..13: note = IgG binding peptide
  SITE 6: note = MISC_FEATURE - X is K, C, D, E, R, V, F, L, 2-Aminooctanedioic acid, Dpr, Orn,AcOrn, AcDab, Dab, Nle, Nva, Tle, Ala(t-Bu), or Cha
DCAYHXGNLVWCT

SEQ ID NO: 18 - protein, 13 aa, synthetic construct
  REGION 1..13: note = IgG binding peptide
  SITE 6: note = MISC_FEATURE - X is K, C, D, E, R, V, F, L, 2-Aminooctanedioic acid, Dpr, Orn,AcOrn, AcDab, Dab, Nle, Nva, Tle, Ala(t-Bu), or Cha
DCTYHXGELVWCT

SEQ ID NO: 19 - protein, 13 aa, synthetic construct
  REGION 1..13: note = IgG binding peptide
  SITE 6: note = MISC_FEATURE - X is K, C, D, E, R, V, F, L, 2-Aminooctanedioic acid, Dpr, Orn,AcOrn, AcDab, Dab, Nle, Nva, Tle, Ala(t-Bu), or Cha
DCAWHXGELVWCT

SEQ ID NO: 20 - protein, 13 aa, synthetic construct
  REGION 1..13: note = IgG binding peptide
  SITE 6: note = MISC_FEATURE - X is K, C, D, E, R, V, F, L, 2-Aminooctanedioic acid, Dpr, Orn,AcOrn, AcDab, Dab, Nle, Nva, Tle, Ala(t-Bu), or Cha
DCTYTXGNLVWCT

SEQ ID NO: 21 - protein, 13 aa, synthetic construct
  REGION 1..13: note = IgG binding peptide
  SITE 6: note = MISC_FEATURE - X is K, C, D, E, R, V, F, L, 2-Aminooctanedioic acid, Dpr, Orn,AcOrn, AcDab, Dab, Nle, Nva, Tle, Ala(t-Bu), or Cha
DCAYTXGNLVWCT

SEQ ID NO: 22 - protein, 13 aa, synthetic construct
  REGION 1..13: note = IgG binding peptide
  SITE 6: note = MISC_FEATURE - X is K, C, D, E, R, V, F, L, 2-Aminooctanedioic acid, Dpr, Orn,AcOrn, AcDab, Dab, Nle, Nva, Tle, Ala(t-Bu), or Cha
DCSYTXGNLVWCT

SEQ ID NO: 23 - protein, 13 aa, synthetic construct
  REGION 1..13: note = IgG binding peptide
  SITE 6: note = MISC_FEATURE - X is K, C, D, E, R, V, F, L, 2-Aminooctanedioic acid, Dpr, Orn,AcOrn, AcDab, Dab, Nle, Nva, Tle, Ala(t-Bu), or Cha
DCTWTXGNLVWCT

SEQ ID NO: 24 - protein, 13 aa, synthetic construct
  REGION 1..13: note = IgG binding peptide
  SITE 6: note = MISC_FEATURE - X is K, C, D, E, R, V, F, L, 2-Aminooctanedioic acid, Dpr, Orn,AcOrn, AcDab, Dab, Nle, Nva, Tle, Ala(t-Bu), or Cha
DCTYHXGNLVWCT

SEQ ID NO: 25 - protein, 13 aa, synthetic construct
  REGION 1..13: note = IgG binding peptide
  SITE 6: note = MISC_FEATURE - X is K, C, D, E, R, V, F, L, 2-Aminooctanedioic acid, Dpr, Orn,AcOrn, AcDab, Dab, Nle, Nva, Tle, Ala(t-Bu), or Cha
DCTYRXGNLVWCT

SEQ ID NO: 26 - protein, 13 aa, synthetic construct
  REGION 1..13: note = IgG binding peptide
  SITE 6: note = MISC_FEATURE - X is K, C, D, E, R, V, F, L, 2-Aminooctanedioic acid, Dpr, Orn,AcOrn, AcDab, Dab, Nle, Nva, Tle, Ala(t-Bu), or Cha
DCTYSXGNLVWCT

SEQ ID NO: 27 - protein, 13 aa, synthetic construct
  REGION 1..13: note = IgG binding peptide
  SITE 6: note = MISC_FEATURE - X is K, C, D, E, R, V, F, L, 2-Aminooctanedioic acid, Dpr, Orn,AcOrn, AcDab, Dab, Nle, Nva, Tle, Ala(t-Bu), or Cha
DCTYTXGNLVWCT

SEQ ID NO: 28 - protein, 13 aa, synthetic construct
  REGION 1..13: note = IgG binding peptide
  SITE 6: note = MISC_FEATURE - X is K, C, D, E, R, V, F, L, 2-Aminooctanedioic acid, Dpr, Orn,AcOrn, AcDab, Dab, Nle, Nva, Tle, Ala(t-Bu), or Cha
DCTYTXGELVWCT

SEQ ID NO: 29 - protein, 13 aa, synthetic construct
  REGION 1..13: note = IgG binding peptide
  SITE 6: note = MISC_FEATURE - X is K, C, D, E, R, V, F, L, 2-Aminooctanedioic acid, Dpr, Orn,AcOrn, AcDab, Dab, Nle, Nva, Tle, Ala(t-Bu), or Cha
DCTYTXGRLVWCT

SEQ ID NO: 30 - protein, 13 aa, synthetic construct
  REGION 1..13: note = IgG binding peptide
  SITE 6: note = MISC_FEATURE - X is K, C, D, E, R, V, F, L, 2-Aminooctanedioic acid, Dpr, Orn,AcOrn, AcDab, Dab, Nle, Nva, Tle, Ala(t-Bu), or Cha
DCTYTXGDLVWCT

SEQ ID NO: 31 - protein, 13 aa, synthetic construct
  REGION 1..13: note = IgG binding peptide
  SITE 6: note = MISC_FEATURE - X is K, C, D, E, R, V, F, L, 2-Aminooctanedioic acid, Dpr, Orn,AcOrn, AcDab, Dab, Nle, Nva, Tle, Ala(t-Bu), or Cha
DCTYTXGNLIWCT

SEQ ID NO: 32 - protein, 13 aa, synthetic construct
  REGION 1..13: note = IgG binding peptide
DCAYHRGELVWCT

SEQ ID NO: 33 - protein, 17 aa, synthetic construct
  REGION 1..17: note = IgG binding peptide
GPDCAYHRGELVWCTFH

SEQ ID NO: 34 - protein, 13 aa, synthetic construct
  REGION 1..13: note = IgG binding peptide
RCAYHRGELVWCS

SEQ ID NO: 35 - protein, 17 aa, synthetic construct
  REGION 1..17: note = IgG binding peptide
GPRCAYHRGELVWCSFH

SEQ ID NO: 36 - protein, 17 aa, synthetic construct
  REGION 1..17: note = IgG binding peptide
SPDCAYHRGELVWCTFH

SEQ ID NO: 37 - protein, 17 aa, synthetic construct
  REGION 1..17: note = IgG binding peptide
GDDCAYHRGELVWCTFH

SEQ ID NO: 38 - protein, 17 aa, synthetic construct
  REGION 1..17: note = IgG binding peptide
GPSCAYHRGELVWCTFH

SEQ ID NO: 39 - protein, 17 aa, synthetic construct
  REGION 1..17: note = IgG binding peptide
GPDCAYHRGELVWCSFH

SEQ ID NO: 40 - protein, 17 aa, synthetic construct
  REGION 1..17: note = IgG binding peptide
GPDCAYHRGELVWCTHH

SEQ ID NO: 41 - protein, 17 aa, synthetic construct
  REGION 1..17: note = IgG binding peptide
GPDCAYHRGELVWCTFY

SEQ ID NO: 42 - protein, 17 aa, synthetic construct
  REGION 1..17: note = IgG binding peptide
SPDCAYHRGELVWCTFY

SEQ ID NO: 43 - protein, 17 aa, synthetic construct
  REGION 1..17: note = IgG binding peptide
SDDCAYHRGELVWCTFY

SEQ ID NO: 44 - protein, 13 aa, synthetic construct
  REGION 1..13: note = IgG binding peptide
DCTYHRGNLVWCT

SEQ ID NO: 45 - protein, 13 aa, synthetic construct
  REGION 1..13: note = IgG binding peptide
DCAYHRGNLVWCT

SEQ ID NO: 46 - protein, 13 aa, synthetic construct
  REGION 1..13: note = IgG binding peptide
DCTYHRGELVWCT

SEQ ID NO: 47 - protein, 13 aa, synthetic construct
  REGION 1..13: note = IgG binding peptide
DCAWHRGELVWCT

SEQ ID NO: 48 - protein, 13 aa, synthetic construct
  REGION 1..13: note = IgG binding peptide
DCTYTNGNLVWCT

SEQ ID NO: 49 - protein, 13 aa, synthetic construct
  REGION 1..13: note = IgG binding peptide
DCAYTNGNLVWCT

SEQ ID NO: 50 - protein, 13 aa, synthetic construct
  REGION 1..13: note = IgG binding peptide
DCSYTNGNLVWCT

SEQ ID NO: 51 - protein, 13 aa, synthetic construct
  REGION 1..13: note = IgG binding peptide
DCTWTNGNLVWCT

SEQ ID NO: 52 - protein, 13 aa, synthetic construct
  REGION 1..13: note = IgG binding peptide
DCTYHNGNLVWCT

SEQ ID NO: 53 - protein, 13 aa, synthetic construct
  REGION 1..13: note = IgG binding peptide
DCTYRNGNLVWCT

SEQ ID NO: 54 - protein, 13 aa, synthetic construct
  REGION 1..13: note = IgG binding peptide
DCTYSNGNLVWCT

SEQ ID NO: 55 - protein, 13 aa, synthetic construct
  REGION 1..13: note = IgG binding peptide
DCTYTRGNLVWCT

SEQ ID NO: 56 - protein, 13 aa, synthetic construct
  REGION 1..13: note = IgG binding peptide
DCTYTNGELVWCT

SEQ ID NO: 57 - protein, 13 aa, synthetic construct
  REGION 1..13: note = IgG binding peptide
DCTYTNGRLVWCT

SEQ ID NO: 58 - protein, 13 aa, synthetic construct
  REGION 1..13: note = IgG binding peptide
DCTYTNGDLVWCT

SEQ ID NO: 59 - protein, 13 aa, synthetic construct
  REGION 1..13: note = IgG binding peptide
DCTYTNGNLIWCT

SEQ ID NO: 60 - protein, 22 aa, synthetic construct
  REGION 1..22: note = IgG binding peptide
GSGGSGPDCAYHRGELVWCTFH

SEQ ID NO: 61 - protein, 18 aa, synthetic construct
  REGION 1..18: note = IgG binding peptide
GSGGSDCAYHRGELVWCT

SEQ ID NO: 62 - protein, 23 aa, synthetic construct
  REGION 1..23: note = IgG binding peptide
KRRRGSGPDCAYHKGELVWCTFH

SEQ ID NO: 63 - protein, 23 aa, synthetic construct
  REGION 1..23: note = IgG binding peptide
KEEGGSGPDCAYHKGELVWCTFH

SEQ ID NO: 64 - protein, 17 aa, synthetic construct
  REGION 1..17: note = IgG binding peptide
GPDCAYHKGELVWCTFH

SEQ ID NO: 65 - protein, 22 aa, synthetic construct
  REGION 1..22: note = IgG binding peptide
RRRGSGPDCAYHKGELVWCTFH

SEQ ID NO: 66 - protein, 22 aa, synthetic construct
  REGION 1..22: note = IgG binding peptide
EEGGSGPDCAYHKGELVWCTFH

SEQ ID NO: 67 - protein, 19 aa, synthetic construct
  REGION 1..19: note = IgG binding peptide
KRRRGSDCAYHKGELVWCT

SEQ ID NO: 68 - protein, 19 aa, synthetic construct
  REGION 1..19: note = IgG binding peptide
KEEGGSDCAYHKGELVWCT

SEQ ID NO: 69 - protein, 13 aa, synthetic construct
  REGION 1..13: note = IgG binding peptide
DCAYHKGELVWCT

SEQ ID NO: 70 - protein, 18 aa, synthetic construct
  REGION 1..18: note = IgG binding peptide
RRRGSDCAYHKGELVWCT

SEQ ID NO: 71 - protein, 18 aa, synthetic construct
  REGION 1..18: note = IgG binding peptide
EEGGSDCAYHKGELVWCT

SEQ ID NO: 72 - protein, 34 aa, synthetic construct
  REGION 1..34: note = IgG binding peptide
FNMQCQRRFYEALHDPNLNEEQRNARIRSIRDDC

SEQ ID NO: 73 - protein, 35 aa, synthetic construct
  REGION 1..35: note = IgG binding peptide
GFNMQCQRRFYEALHDPNLNEEQRNARIRSIRDDC

SEQ ID NO: 74 - protein, 34 aa, synthetic construct
  REGION 1..34: note = IgG binding peptide
KNMQCQRRFYEALHDPNLNEEQRNARIRSIRDDC

SEQ ID NO: 75 - protein, 35 aa, synthetic construct
  REGION 1..35: note = IgG binding peptide
GFNMQCQKRFYEALHDPNLNEEQRNARIRSIRDDC

SEQ ID NO: 76 - protein, 34 aa, synthetic construct
  REGION 1..34: note = IgG binding peptide
KNMQCQKRFYEALHDPNLNEEQRNARIRSIRDDC

SEQ ID NO: 77 - protein, 33 aa, synthetic construct
  REGION 1..33: note = IgG binding peptide
FNMQQQRRFYEALHDPNLNEEQRNARIRSIRDD

SEQ ID NO: 78 - protein, 35 aa, synthetic construct
  REGION 1..35: note = IgG binding peptide
GKNMQCQRRFYEALHDPNLNEEQRNARIRSIRDDC

SEQ ID NO: 79 - protein, 40 aa, synthetic construct
  REGION 1..40: note = IgG binding peptide
FNMQQQRRFYEALHDPNLNEEQRNARIRSIRDDPSGSGSK

SEQ ID NO: 80 - protein, 40 aa, synthetic construct
  REGION 1..40: note = IgG binding peptide
FNMQCQRRFYEALHDPNLNEEQRNARIRSIRDDCSGSGSK

SEQ ID NO: 81 - protein, 34 aa, synthetic construct
  REGION 1..34: note = IgG binding peptide
FNMQQQRRFYEALHDPNLNEEQRNARIRSIRDDP

SEQ ID NO: 82 - protein, 33 aa, synthetic construct
  REGION 1..33: note = IgG binding peptide
FNMQQQCRFYEALHDPNLNEEQRNARIRSIRDD

SEQ ID NO: 83 - protein, 34 aa, synthetic construct
  REGION 1..34: note = IgG binding peptide
FNMQQQRRFYEALHDPNLNEEQRNARIRSIRDDC

SEQ ID NO: 84 - protein, 39 aa, synthetic construct
  REGION 1..39: note = IgG binding peptide
FNMQQQRRFYEALHDPNLNEEQRNARIRSIRDDPSRRKR

SEQ ID NO: 85 - protein, 39 aa, synthetic construct
  REGION 1..39: note = IgG binding peptide
FNMQQQRRFYEALHDPNLNEEQRNARIRSIRDDPSRRCR

SEQ ID NO: 86 - protein, 44 aa, synthetic construct
  REGION 1..44: note = IgG binding peptide
FNMQQQCRFYEALHDPNLNEEQRNARICSIRDDPSRRCRRCRRC

SEQ ID NO: 87 - protein, 44 aa, synthetic construct
  REGION 1..44: note = IgG binding peptide
FNMQQQKRFYEALHDPNLNEEQRNARIKSIRDDPSRRKRRKRRK

SEQ ID NO: 88 - protein, 33 aa, synthetic construct
  REGION 1..33: note = IgG binding peptide
KNMQQQCRFYEALHDPNLNEEQRNARIRSIRDD

SEQ ID NO: 89 - protein, 34 aa, synthetic construct
  REGION 1..34: note = IgG binding peptide
KNMQQQRRFYEALHDPNLNEEQRNARIRSIRDDC

SEQ ID NO: 90 - protein, 39 aa, synthetic construct
  REGION 1..39: note = IgG binding peptide
KNMQQQRRFYEALHDPNLNEEQRNARIRSIRDDPSRRKR

SEQ ID NO: 91 - protein, 39 aa, synthetic construct
  REGION 1..39: note = IgG binding peptide
KNMQQQRRFYEALHDPNLNEEQRNARIRSIRDDPSRRCR

SEQ ID NO: 92 - protein, 44 aa, synthetic construct
  REGION 1..44: note = IgG binding peptide
KNMQQQCRFYEALHDPNLNEEQRNARICSIRDDPSRRCRRCRRC

SEQ ID NO: 93 - protein, 44 aa, synthetic construct
  REGION 1..44: note = IgG binding peptide
KNMQQQKRFYEALHDPNLNEEQRNARIKSIRDDPSRRKRRKRRK

SEQ ID NO: 94 - protein, 34 aa, synthetic construct
  REGION 1..34: note = IgG binding peptide
GFNMQQQCRFYEALHDPNLNEEQRNARIRSIRDD

SEQ ID NO: 95 - protein, 35 aa, synthetic construct
  REGION 1..35: note = IgG binding peptide
GFNMQQQRRFYEALHDPNLNEEQRNARIRSIRDDC

SEQ ID NO: 96 - protein, 40 aa, synthetic construct
  REGION 1..40: note = IgG binding peptide
GFNMQQQRRFYEALHDPNLNEEQRNARIRSIRDDPSRRKR

SEQ ID NO: 97 - protein, 40 aa, synthetic construct
  REGION 1..40: note = IgG binding peptide
GFNMQQQRRFYEALHDPNLNEEQRNARIRSIRDDPSRRCR

SEQ ID NO: 98 - protein, 45 aa, synthetic construct
  REGION 1..45: note = IgG binding peptide
GFNMQQQCRFYEALHDPNLNEEQRNARICSIRDDPSRRCRRCRRC

SEQ ID NO: 99 - protein, 45 aa, synthetic construct
  REGION 1..45: note = IgG binding peptide
GFNMQQQKRFYEALHDPNLNEEQRNARIKSIRDDPSRRKRRKRRK

SEQ ID NO: 100 - protein, 34 aa, synthetic construct
  REGION 1..34: note = IgG binding peptide
FNMQCQZRFYEALHDPNLNEEQRNARIRSIRDDC

SEQ ID NO: 101 - protein, 34 aa, synthetic construct
  REGION 1..34: note = IgG binding peptide
KNMQCQZRFYEALHDPNLNEEQRNARIRSIRDDC

SEQ ID NO: 102 - protein, 40 aa, synthetic construct
  REGION 1..40: note = IgG binding peptide
GFNMQCQKRFYEALHDPNLNEEQRNARIRSIRDDCSRRKR

SEQ ID NO: 103 - protein, 34 aa, synthetic construct
  REGION 1..34: note = IgG binding peptide
FNMQCQKRFYEALHDPNLNEEQRNARIRSIRDDC

SEQ ID NO: 104 - protein, 39 aa, synthetic construct
  REGION 1..39: note = IgG binding peptide
KNMQCQKRFYEALHDPNLNEEQRNARIRSIRDDCSRRKR

SEQ ID NO: 105 - protein, 45 aa, synthetic construct
  REGION 1..45: note = IgG binding peptide
GFNMQCQKRFYEALHDPNLNEEQRNARIRSIRDDCSRRKRRKRRK

SEQ ID NO: 106 - protein, 44 aa, synthetic construct
  REGION 1..44: note = IgG binding peptide
KNMQCQKRFYEALHDPNLNEEQRNARIRSIRDDCSRRKRRKRRK

SEQ ID NO: 107 - protein, 45 aa, synthetic construct; identical to SEQ ID NO: 105
  REGION 1..45: note = IgG binding peptide

SEQ ID NO: 108 - protein, 11 aa, synthetic construct
  REGION 1..11: note = IgG binding peptide
CAWHLGELVWC

SEQ ID NO: 109 - protein, 13 aa, synthetic construct
  REGION 1..13: note = IgG binding peptide
DCAWHLGELVWCT

SEQ ID NO: 110 - protein, 13 aa, synthetic construct
  REGION 1..13: note = IgG binding peptide
DCAWHLGELVFCT

SEQ ID NO: 111 - protein, 13 aa, synthetic construct
  REGION 1..13: note = IgG binding peptide
  SITE 11: note = MISC_FEATURE - X is 1-naphtoyl, 2-naphtoyl, benzyl, or benzothiophene
DCAWHLGELVXCT

SEQ ID NO: 112 - protein, 15 aa, synthetic construct
  REGION 1..15: note = IgG binding peptide
CDCAWHLGELVWCTC

SEQ ID NO: 113 - protein, 11 aa, synthetic construct
  REGION 1..11: note = IgG binding peptide
CAYHLGELVWC

SEQ ID NO: 114 - protein, 14 aa, synthetic construct
  REGION 1..14: note = IgG binding peptide
DCAYHLGELVWCTF

SEQ ID NO: 115 - protein, 23 aa, synthetic construct
  REGION 1..23: note = IgG binding peptide
KRRRGSGPDCAYHKGELVWCTFH

SEQ ID NO: 116 - protein, 33 aa, synthetic construct
  REGION 1..33: note = IgG binding peptide
NMQCQRRFYEALHDPNLNEEQRNARIRSIRDDC

SEQ ID NO: 117 - protein, 34 aa, synthetic construct; identical to SEQ ID NO: 72
  REGION 1..34: note = IgG binding peptide

SEQ ID NO: 118 - protein, 33 aa, synthetic construct; identical to SEQ ID NO: 116
  REGION 1..33: note = IgG binding peptide

SEQ ID NO: 119 - protein, 34 aa, synthetic construct; identical to SEQ ID NO: 103
  REGION 1..34: note = IgG binding peptide

SEQ ID NO: 120 - protein, 33 aa, synthetic construct
  REGION 1..33: note = IgG binding peptide
NMQCQKRFYEALHDPNLNEEQRNARIRSIRDDC

SEQ ID NO: 121 - protein, 32 aa, synthetic construct
  REGION 1..32: note = IgG binding peptide
NMQQQRRFYEALHDPNLNEEQRNARIRSIRDD

SEQ ID NO: 122 - protein, 34 aa, synthetic construct; identical to SEQ ID NO: 74
  REGION 1..34: note = IgG binding peptide

SEQ ID NO: 123 - protein, 39 aa, synthetic construct
  REGION 1..39: note = IgG binding peptide
NMQQQRRFYEALHDPNLNEEQRNARIRSIRDDPSGSGSK

SEQ ID NO: 124 - protein, 39 aa, synthetic construct
  REGION 1..39: note = IgG binding peptide
NMQCQRRFYEALHDPNLNEEQRNARIRSIRDDCSGSGSK

SEQ ID NO: 125 - protein, 33 aa, synthetic construct
  REGION 1..33: note = IgG binding peptide
NMQQQRRFYEALHDPNLNEEQRNARIRSIRDDP

SEQ ID NO: 126 - protein, 32 aa, synthetic construct
  REGION 1..32: note = IgG binding peptide
NMQQQCRFYEALHDPNLNEEQRNARIRSIRDD

SEQ ID NO: 127 - protein, 33 aa, synthetic construct
  REGION 1..33: note = IgG binding peptide
NMQQQRRFYEALHDPNLNEEQRNARIRSIRDDC

SEQ ID NO: 128 - protein, 38 aa, synthetic construct
  REGION 1..38: note = IgG binding peptide
NMQQQRRFYEALHDPNLNEEQRNARIRSIRDDPSRRKR

SEQ ID NO: 129 - protein, 38 aa, synthetic construct
  REGION 1..38: note = IgG binding peptide
NMQQQRRFYEALHDPNLNEEQRNARIRSIRDDPSRRCR

SEQ ID NO: 130 - protein, 43 aa, synthetic construct
  REGION 1..43: note = IgG binding peptide
NMQQQCRFYEALHDPNLNEEQRNARICSIRDDPSRRCRRCRRC

SEQ ID NO: 131 - protein, 43 aa, synthetic construct
  REGION 1..43: note = IgG binding peptide
NMQQQKRFYEALHDPNLNEEQRNARIKSIRDDPSRRKRRKRRK

SEQ ID NO: 132 - protein, 32 aa, synthetic construct; identical to SEQ ID NO: 126
  REGION 1..32: note = IgG binding peptide

SEQ ID NO: 133 - protein, 33 aa, synthetic construct; identical to SEQ ID NO: 127
  REGION 1..33: note = IgG binding peptide

SEQ ID NO: 134 - protein, 38 aa, synthetic construct; identical to SEQ ID NO: 128
  REGION 1..38: note = IgG binding peptide

SEQ ID NO: 135 - protein, 38 aa, synthetic construct; identical to SEQ ID NO: 129
  REGION 1..38: note = IgG binding peptide

SEQ ID NO: 136 - protein, 43 aa, synthetic construct; identical to SEQ ID NO: 130
  REGION 1..43: note = IgG binding peptide

SEQ ID NO: 137 - protein, 43 aa, synthetic construct; identical to SEQ ID NO: 131
  REGION 1..43: note = IgG binding peptide

SEQ ID NO: 138 - protein, 33 aa, synthetic construct; identical to SEQ ID NO: 82
  REGION 1..33: note = IgG binding peptide

SEQ ID NO: 139 - protein, 34 aa, synthetic construct; identical to SEQ ID NO: 83
  REGION 1..34: note = IgG binding peptide

SEQ ID NO: 140 - protein, 39 aa, synthetic construct; identical to SEQ ID NO: 84
  REGION 1..39: note = IgG binding peptide

SEQ ID NO: 141 - protein, 39 aa, synthetic construct; identical to SEQ ID NO: 85
  REGION 1..39: note = IgG binding peptide

SEQ ID NO: 142 - protein, 44 aa, synthetic construct; identical to SEQ ID NO: 86
  REGION 1..44: note = IgG binding peptide

SEQ ID NO: 143 - protein, 44 aa, synthetic construct; identical to SEQ ID NO: 87
  REGION 1..44: note = IgG binding peptide

SEQ ID NO: 144 - protein, 33 aa, synthetic construct
  REGION 1..33: note = IgG binding peptide
NMQCQZRFYEALHDPNLNEEQRNARIRSIRDDC

SEQ ID NO: 145 - protein, 33 aa, synthetic construct; identical to SEQ ID NO: 144
  REGION 1..33: note = IgG binding peptide

SEQ ID NO: 146 - protein, 39 aa, synthetic construct
  REGION 1..39: note = IgG binding peptide
FNMQCQKRFYEALHDPNLNEEQRNARIRSIRDDCSRRKR

SEQ ID NO: 147 - protein, 33 aa, synthetic construct; identical to SEQ ID NO: 120
  REGION 1..33: note = IgG binding peptide

SEQ ID NO: 148 - protein, 38 aa, synthetic construct
  REGION 1..38: note = IgG binding peptide
NMQCQKRFYEALHDPNLNEEQRNARIRSIRDDCSRRKR

SEQ ID NO: 149 - protein, 44 aa, synthetic construct
  REGION 1..44: note = IgG binding peptide
FNMQCQKRFYEALHDPNLNEEQRNARIRSIRDDCSRRKRRKRRK

SEQ ID NO: 150 - protein, 43 aa, synthetic construct
  REGION 1..43: note = IgG binding peptide
NMQCQKRFYEALHDPNLNEEQRNARIRSIRDDCSRRKRRKRRK

SEQ ID NO: 151 - protein, 44 aa, synthetic construct; identical to SEQ ID NO: 149
  REGION 1..44: note = IgG binding peptide

SEQ ID NO: 152 - protein, 33 aa, synthetic construct; identical to SEQ ID NO: 116
  REGION 1..33: note = IgG binding peptide
  DISULFID 4..33: note = intrachain disulfide bond
  MOD_RES 1: note = hydrogen atom of amino group is replaced
  MOD_RES 33: note = carboxyl group is amidated

SEQ ID NO: 153 - protein, 17 aa, synthetic construct
  DISULFID 4..14: note = intrachain disulfide bond
  REGION 1..17: note = IgG binding peptide
  MOD_RES 17: note = carboxyl group is amidated
  MOD_RES 8: note = amino group of side-chain end is modified
  MOD_RES 1: note = N-terminal is modified
GPDCAYHKGELVWCTFH

SEQ ID NO: 154 - protein, 22 aa, synthetic construct
GSGGSGPDCAYHRGELVWCTFH

SEQ ID NO: 155 - protein, 13 aa, synthetic construct
XCXXXXGXLXWCX

SEQ ID NO: 156 - protein, 5 aa, synthetic construct
RRRGS

SEQ ID NO: 157 - protein, 5 aa, synthetic construct
EEGGS

SEQ ID NO: 158 - protein, 5 aa, synthetic construct
GSGGS

SEQ ID NO: 159 - protein, 10 aa, synthetic construct
GSGGSGSGGS

SEQ ID NO: 160 - protein, 15 aa, synthetic construct
GSGGSGSGGSGSGGS

SEQ ID NO: 161 - protein, 5 aa, synthetic construct
SGSGS

SEQ ID NO: 162 - protein, 10 aa, synthetic construct
SGSGSSGSGS

SEQ ID NO: 163 - protein, 15 aa, synthetic construct
SGSGSSGSGSSGSGS

SEQ ID NO: 164 - protein, 6 aa, synthetic construct
SGSGSK

SEQ ID NO: 165 - protein, 5 aa, synthetic construct
SRRCR

SEQ ID NO: 166 - protein, 5 aa, synthetic construct
  MOD_RES 4: note = a functional group-bonded lysine residue
SRRKR

SEQ ID NO: 167 - protein, 10 aa, synthetic construct
SRRCRRCRRC

SEQ ID NO: 168 - protein, 10 aa, synthetic construct
  MOD_RES 4: note = a functional group-bonded lysine residue
  MOD_RES 7: note = a functional group-bonded lysine residue
  MOD_RES 10: note = a functional group-bonded lysine residue
SRRKRRKRRK